European Patent Specification EP 4 399 327 B1, published October 29, 2025. Title: NON-SEQUENCING PCR-BASED METHOD FOR DETECTION OF ANTIBODY-CONJUGATED OLIGONUCLEOTIDES. Applicant: Becton, Dickinson and Company. The sequence listing filed with the application follows.

SEQUENCE LISTING (9 sequences)

SEQ ID NO: 1 - DNA, 95 bp, synthetic construct
  misc_feature <1: note = 5'AmMC6 - 5' Amino Modifier C6
  source 1..95: mol_type = other DNA
gttgtcaagatgctaccgttcagagtacgtggagttggtggcccgaccccgagcgctacgagccccccggaaaaaaaaaaaaaaaaaaaaaaaaa

SEQ ID NO: 2 - DNA, 200 bp, synthetic construct
  misc_feature <1: note = 5AmMC6 - 5' Amino Modifier C6
  source 1..200: mol_type = other DNA
gttgtcaagatgctaccgttcagagctactgtccgaagttaccgtgtatctaccacgggtggtttttcgaatccggaaaagatagtaataagtgttttagttggaataagtcgcaacttttggagacggttacctctcaatttttctgatccgtaggccccccgatctcggcctcaaaaaaaaaaaaaaaaaaaaaaaaa

SEQ ID NO: 3 - DNA, 25 bp, synthetic construct
  source 1..25: mol_type = other DNA
gttgtcaagatgctaccgttcagag

SEQ ID NO: 4 - DNA, 20 bp, synthetic construct
  source 1..20: mol_type = other DNA
acacgacgctcttccgatct

SEQ ID NO: 5 - DNA, 95 bp, synthetic construct
  source 1..95: mol_type = other DNA
gttgtcaagatgctaccgttcagagccccatgtctagtacctattggtcccctatcctcagattcgtttaaaaaaaaaaaaaaaaaaaaaaaaaa

SEQ ID NO: 6 - DNA, 26 bp, synthetic construct
  source 1..26: mol_type = other DNA
tttttttttttttttttttttttttt

SEQ ID NO: 7 - DNA, 95 bp, synthetic construct
  misc_feature <1: note = 5AmMC12 - 5' Amino Modifier C12
  source 1..95: mol_type = other DNA
gttgtcaagatgctaccgttcagagattcaagggcagccgcgtcacgattggatacgactgttggaccggaaaaaaaaaaaaaaaaaaaaaaaaa

SEQ ID NO: 8 - DNA, 102 bp, synthetic construct
  misc_feature <1: note = 5'AmMC12 - 5' Amino Modifier C12
  source 1..102: mol_type = other DNA
cagacgtgtgctcttccgatctvnnvnnnnvnnvnnnnnnnnnnnnnnnnnnnnnnnnnnnnnnnnnnnnnnnnnbbaaaaaaaaaaaaaaaaaaaaaaaaa

SEQ ID NO: 9 - DNA, 10 bp, synthetic construct
  source 1..10: mol_type = other DNA
aaaaaaaaaa